European Patent Application EP 4 253 561 A1, published October 4, 2023. Title: METHOD FOR PRODUCING COMPLEX, METHOD FOR DETERMINING MICROBIAL INCLUSION, AND METHOD FOR IDENTIFYING INCLUDED MICROORGANISM. Applicant: Yokogawa Electric Corporation. The sequence listing filed with the application follows.

SEQUENCE LISTING (9 sequences)

SEQ ID NO: 1 - DNA, 445 bp, synthetic construct
  misc_feature 1..445: note = synthetic
  source 1..445: mol_type = other DNA
cttgttacgacttcaccccagtcatgaatcacaaagtggtaagcgccctcccgaaggttaagctacctacttcttttgcaacccactcccatggtgtgacgggcggtgtgtacaaggcccgggaacgtattcaccgtggcattctgatccacgattactagcgattccgacttcatggagtcgagttgcagactccaatccggactacgacgcactttatgaggtccgcttgctctcgcgaggtcgcttctctttgtatgcgccattgtagcacgtgtgtagccctggtcgtaagggccatgatgacttgacgtcatccccaccttcctccagtttatcactggcagtctcctttgagttcccggccggaccgctggcaacaaaggataagggttgcgctcgttgcgggacttaacccaacatttcacaacacgagctgacgaca

SEQ ID NO: 2 - DNA, 48 bp, synthetic construct
  misc_feature 1..48: note = probe
  source 1..48: mol_type = other DNA
actcaaaggagactgccagtgataaactggagcagtgataaactggag

SEQ ID NO: 3 - DNA, 48 bp, synthetic construct
  misc_feature 1..48: note = probe
  source 1..48: mol_type = other DNA
gcagtctcctttgagtgcagtctcctttgagtctccagtttatcactg

SEQ ID NO: 4 - DNA, 24 bp, synthetic construct
  misc_feature 1..24: note = probe
  source 1..24: mol_type = other DNA
gaatcgctagtaatcgtggatcag

SEQ ID NO: 5 - DNA, 16 bp, synthetic construct
  misc_feature 1..16: note = probe
  source 1..16: mol_type = other DNA
actcaaaggagactgc

SEQ ID NO: 6 - DNA, 16 bp, synthetic construct
  misc_feature 1..16: note = probe
  source 1..16: mol_type = other DNA
cagtgataaactggag

SEQ ID NO: 7 - DNA, 24 bp, synthetic construct
  misc_feature 1..24: note = probe
  source 1..24: mol_type = other DNA
aaaggagactgccagtgataaact

SEQ ID NO: 8 - DNA, 16 bp, synthetic construct
  misc_feature 1..16: note = probe
  source 1..16: mol_type = other DNA
gcagtctcctttgagt

SEQ ID NO: 9 - DNA, 16 bp, synthetic construct
  misc_feature 1..16: note = probe
  source 1..16: mol_type = other DNA
ctccagtttatcactg